European Patent Application EP 4 374 852 A2, published May 29, 2024. Title: Anti-CDH6 antibody and anti-CDH6 antibody-drug conjugate. Applicant: DAIICHI SANKYO COMPANY, LIMITED. Application EP. The sequence listing filed with the application follows.

SEQUENCE LISTING (86 sequences)

SEQ ID NO: 1 - protein, 790 aa, Homo sapiens
MRTYRYFLLLFWVGQPYPTLSTPLSKRTSGFPAKKRALELSGNSKNELNRSKRSWMWNQFFLLEEYTGSDYQYVGKLHSDQDRGDGSLKYILSGDGAGDLFIINENTGDIQATKRLDREEKPVYILRAQAINRRTGRPVEPESEFIIKIHDINDNEPIFTKEVYTATVPEMSDVGTFVVQVTATDADDPTYGNSAKVVYSILQGQPYFSVESETGIIKTALLNMDRENREQYQVVIQAKDMGGQMGGLSGTTTVNITLTDVNDNPPRFPQSTYQFKTPESSPPGTPIGRIKASDADVGENAEIEYSITDGEGLDMFDVITDQETQEGIITVKKLLDFEKKKVYTLKVEASNPYVEPRFLYLGPFKDSATVRIVVEDVDEPPVFSKLAYILQIREDAQINTTIGSVTAQDPDAARNPVKYSVDRHTDMDRIFNIDSGNGSIFTSKLLDRETLLWHNITVIATEINNPKQSSRVPLYIKVLDVNDNAPEFAEFYETFVCEKAKADQLIQTLHAVDKDDPYSGHQFSFSLAPEAASGSNFTIQDNKDNTAGILTRKNGYNRHEMSTYLLPVVISDNDYPVQSSTGTVTVRVCACDHHGNMQSCHAEALIHPTGLSTGALVAILLCIVILLVTVVLFAALRRQRKKEPLIISKEDIRDNIVSYNDEGGGEEDTQAFDIGTLRNPEAIEDNKLRRDIVPEALFLPRRTPTARDNTDVRDFINQRLKENDTDPTAPPYDSLATYAYEGTGSVADSLSSLESVTTDADQDYDYLSDWGPRFKKLADMYGGVDSDKDS

SEQ ID NO: 2 - protein, 106 aa, Homo sapiens
SWMWNQFFLLEEYTGSDYQYVGKLHSDQDRGDGSLKYILSGDGAGDLFIINENTGDIQATKRLDREEKPVYILRAQAINRRTGRPVEPESEFIIKIHDINDNEPIF

SEQ ID NO: 3 - protein, 109 aa, Homo sapiens
TKEVYTATVPEMSDVGTFVVQVTATDADDPTYGNSAKVVYSILQGQPYFSVESETGIIKTALLNMDRENREQYQVVIQAKDMGGQMGGLSGTTTVNITLTDVNDNPPRF

SEQ ID NO: 4 - protein, 115 aa, Homo sapiens
PQSTYQFKTPESSPPGTPIGRIKASDADVGENAEIEYSITDGEGLDMFDVITDQETQEGIITVKKLLDFEKKKVYTLKVEASNPYVEPRFLYLGPFKDSATVRIVVEDVDEPPVF

SEQ ID NO: 5 - protein, 103 aa, Homo sapiens
SKLAYILQIREDAQINTTIGSVTAQDPDAARNPVKYSVDRHTDMDRIFNIDSGNGSIFTSKLLDRETLLWHNITVIATEINNPKQSSRVPLYIKVLDVNDNAP

SEQ ID NO: 6 - protein, 122 aa, Homo sapiens
EFAEFYETFVCEKAKADQLIQTLHAVDKDDPYSGHQFSFSLAPEAASGSNFTIQDNKDNTAGILTRKNGYNRHEMSTYLLPVVISDNDYPVQSSTGTVTVRVCACDHHGNMQSCHAEALIHP

SEQ ID NO: 7 - protein, 790 aa, Mus musculus
MRTYRYFLLLFWVGQPYPTFSNPLSKRTSGFPAKRKALELSANSRNELSRSKRSWMWNQFFLLEEYTGSDYQYVGKLHSDQDRGDGSLKYILSGDGAGDLFIINENTGDIQATKRLDREEKPVYILRAQAVNRRTGRPVEPESEFIIKIHDINDNEPIFTKDVYTATVPEMADVGTFVVQVTATDADDPTYGNSAKVVYSILQGQPYFSVESETGIIKTALLNMDRENREQYQVVIQAKDMGGQMGGLSGTTTVNITLTDVNDNPPRFPQSTYQFKTPESSPPGTPIGRIKASDADVGENAEIEYSITDGEGHEMFDVITDQETQEGIITVKKLLDFEKKKVYTLKVEASNPHVEPRFLYLGPFKDSATVRIVVDDVDEPPVFSKLAYILQIREDARINTTIGSVAAQDPDAARNPVKYSVDRHTDMDRIFNIDSGNGSIFTSKLLDRETLLWHNITVIATEINNPKQSSRVPLYIKVLDVNDNAPEFAEFYETFVCEKAKADQLIQTLRAVDKDDPYSGHQFSFSLAPEAASSSNFTIQDNKDNTAGILTRKNGYNRHEMSTYLLPVVISDNDYPVQSSTGTVTVRVCACDHHGNMQSCHAEALIHPTGLSTGALVAILLCIVILLVTVVLFAALRRQRKKEPLIISKEDIRDNIVSYNDEGGGEEDTQAFDIGTLRNPEAMEDSKSRRDIVPEALFLPRRTPTARDNTDVRDFINQRLKENDTDPTAPPYDSLATYAYEGTGSVADSLSSLESVTTDGDQDYDYLSDWGPRFKKLADMYGGMDSDKDS

SEQ ID NO: 8 - protein, 789 aa, Rattus norvegicus
MRTYRYFLLLFWVGQPYPTFSNPLSKRTSGFPAKRRALELSANSRNELSRSKRSWMWNQFFLLEEYTGSDYQYVGKLHSDQDRGDGSLKYILSGDGAGDLFIINENTGDIQATKRLDREEKPVYILRAQAINRRTGRPVEPESEFIIKIHDINDNEPIFTKDVYTATVPEMADVGTFVVQVTATDADDPTYGNSAKVVYSILQGQPYFSVESETGIIKTALLNMDRENREQYQVVIQAKDMGGQMGGLSGTTTVNITLTDVNDNPPRFPQSTYQFKTPESSPPGTPIGRIKASDADVGENAEIEYSITDGEGHDMFDVITDQETQEGIITVKKLLDFEKKRVYTLKVEASNPHIEPRFLYLGPFKDSATVRIVVDDVDEPPVFSKPAYILQIREDAQINTTIGSVAAQDPDAARNPVKYSVDRHTDMDRIFNIDSGNGSIFTSKLLDRETLLWHNITVIATEINNPKQSSRVPLYIKVLDVNDNAPEFAEFYETFVCEKAKADQLIQTLHAVDKDDPYSGHQFSFSLAPEAASGSNFTIQDNKDNTAGILTRKNGYNRHEMSTYLLPVVISDNDYPVQSSTGTVTVRVCACDHHGNMQSCHAEALIHPTGLSTGALVAILLCIVILLVTVVLFAALRRQRKKEPLIISKEDIRDNIVSYNDEGGGEEDTQAFDIGTLRNPKPWRQQSRRDMVPEALFLPRRTPTARDNTDVRDFISQRLRKMNTDPTAPPYDSLATYAYEGTGSVADSLSSLESVTTDGDQDYGYLSDWGPRFKKLADMYGGMDSDKDS

SEQ ID NO: 9 - protein, 790 aa, Macaca fascicularis
MRTYRYFLLLFWVGQPYPTLSTPLSKRTSGFPAKKRALELSGNSKNELNRSKRSWMWNQFFLLEEYTGSDYQYVGKLHSDQDRGDGSLKYILSGDGAGDLFIINENTGDIQATKRLDREEKPVYILRAQAINRRTGRPVEPESEFIIKIHDINDNEPIFTKEVYTATVPEMSDVGTFVVQVTATDADDPTYGNSAKVVYSILQGQPYFSVESETGIIKTALLNMDRENREQYQVVIQAKDMGGQMGGLSGTTTVNITLTDVNDNPPRFPQSTYQFKTPESSPPGTPIGRIKASDADVGENAEIEYSITDGEGLDMFDVITDQETQEGIITVKKLLDFEKKKVYTLKVEASNPHVEPRFLYLGPFKDSATVRIVVEDVDEPPVFSKLAYILQIREDAQINTTIGSVTAQDPDAARNPVKYSVDRHTDMDRIFNIDSGNGSIFTSKLLDRETLLWHNITVIATEINNPKQSSRVPLYIKVLDVNDNAPEFAEFYETFVCEKAKADQLIQTLRAVDKDDPYSGHQFSFSLAPEAASGSNFTIQDNKDNTAGILTRKNGYNRHEMSTYLLPVVISDNDYPVQSSTGTVTVRVCACDHHGNMQSCHAEALIHPTGLSTGALVAILLCIVILLVTVVLFAALRRQRKKEPLIISKEDIRDNIVSYNDEGGGEEDTQAFDIGTLRNPEAIEDNKLRRDIVPEALFLPRRTPTARDNTDVRDFINQRLKENDTDPTAPPYDSLATYAYEGTGSVADSLSSLESVTTDGDQDYDYLSDWGPRFKKLADMYGGVDSDKDS

SEQ ID NO: 10 - protein, 108 aa, Rattus norvegicus
DIQMTQSPSLLSASVGDRVTLNCKASQNIYKNLAWYQQKLGEGPKLLIYDANTLQTGIPSRFSGSGSGSDFTLTISSLQPEDVATYFCQQYYSGWAFGGVTNLELKRA

SEQ ID NO: 11 - DNA, 324 bp, Rattus norvegicus
  source 1..324: mol_type = genomic DNA
gacatccagatgacccagtctccttcactcctgtctgcatctgtgggagacagagtcactctcaactgcaaagcaagtcagaatatttataagaacttagcctggtatcagcaaaagcttggagaaggtcccaaactcctgatttatgatgcaaacactttgcaaacgggcatcccatcaaggttcagtggcagtggatctggttcagatttcacactcaccatcagcagcctgcagcctgaagatgttgccacatatttctgccagcagtactatagcgggtgggcgttcggtggagtcaccaacctggaattgaaacgggct

SEQ ID NO: 12 - protein, 11 aa, Rattus norvegicus
KASQNIYKNLA

SEQ ID NO: 13 - protein, 7 aa, Rattus norvegicus
DANTLQT

SEQ ID NO: 14 - protein, 8 aa, Rattus norvegicus
QQYYSGWA

SEQ ID NO: 15 - protein, 122 aa, Rattus norvegicus
QVQLQQSGAELVKPGSSVKISCKASGYTFTRNFMHWIKQQPGNGLEWIGWIYCGDGETEYNQKFNGKATLTADRSSSTAYMELSRLTSEDSAVYFCARGVYGGFAGGYFDFWGQGVMVTVSS

SEQ ID NO: 16 - DNA, 366 bp, Rattus norvegicus
  source 1..366: mol_type = genomic DNA
caggtacagctgcagcaatctggggctgaactggtgaagcctgggtcctcagtgaaaatttcctgcaaggcttctggctacaccttcaccaggaactttatgcactggataaaacagcagcctggaaatggccttgagtggattgggtggatttattgtggagatggtgagacagagtacaatcaaaagttcaatgggaaggcaacactcactgcggacagatcctccagcacagcctatatggagctcagcagactgacatctgaggactctgcagtctatttctgtgcaagaggggtttacggagggtttgccgggggctactttgatttctggggccaaggagtcatggtcacagtctcctca

SEQ ID NO: 17 - protein, 10 aa, Rattus norvegicus
GYTFTRNFMH

SEQ ID NO: 18 - protein, 10 aa, Rattus norvegicus
WIYCGDGETE

SEQ ID NO: 19 - protein, 13 aa, Rattus norvegicus
GVYGGFAGGYFDF

SEQ ID NO: 20 - protein, 109 aa, Rattus norvegicus
DVQMTHSPSYLAASPGESVSISCKTSKNISNYLVWYQQKPGEAYKLLIYSGSTLQSGTPSRFSGSGSGTDFTLTIRSLEPEDFGLYFCQQYYEKPFTFGSGTKLEIKRA

SEQ ID NO: 21 - DNA, 327 bp, Rattus norvegicus
  source 1..327: mol_type = genomic DNA
gatgtccagatgacccactctccgtcttatcttgctgcgtctcctggagaaagtgtttccatcagttgcaagacaagtaagaacattagtaattatttagtctggtatcaacagaaacctggggaagcatataagcttcttatctattctgggtcaactttgcaatctggaactccatcaaggttcagtggcagtggatctggtacagatttcactctcactatcagaagcctggagcctgaagattttggactctatttctgtcaacagtattatgaaaaaccattcacgttcggctcagggacgaagttggaaataaaacgggct

SEQ ID NO: 22 - protein, 11 aa, Rattus norvegicus
KTSKNISNYLV

SEQ ID NO: 23 - protein, 7 aa, Rattus norvegicus
SGSTLQS

SEQ ID NO: 24 - protein, 9 aa, Rattus norvegicus
QQYYEKPFT

SEQ ID NO: 25 - protein, 121 aa, Rattus norvegicus
EVQLQESGPGLVRPSQSLSLSCSVTDYSITSNYWGWIRRFPGNKMEWMGYITYSGYTSYNPSLQSRISITRDTSKNQFFLQLNSVTAEDTATYYCARSINHGGYSYVVDAWGPGASVTVSS

SEQ ID NO: 26 - DNA, 363 bp, Rattus norvegicus
  source 1..363: mol_type = genomic DNA
gaggtgcaacttcaggagtcaggacctggccttgtgagaccctcacagtcactctccctctcctgttctgtcactgattactccatcactagtaattactggggctggatccggaggttcccaggaaataaaatggagtggatgggatacataacctatagtggttacactagctacaacccatctctccaaagtcgaatctccattactagagacacatcgaagaatcagttcttcctgcagttgaactctgtaactgctgaggacacagccacatattactgtgcaagatcgattaaccacggaggatatagttatgttgtggatgcctggggtccgggagcttcagtcactgtctcctca

SEQ ID NO: 27 - protein, 10 aa, Rattus norvegicus
DYSITSNYWG

SEQ ID NO: 28 - protein, 9 aa, Rattus norvegicus
YITYSGYTS

SEQ ID NO: 29 - protein, 13 aa, Rattus norvegicus
SINHGGYSYVVDA

SEQ ID NO: 30 - protein, 109 aa, Rattus norvegicus
DVQMTQSPSSLAASPGESVSISCRATKSIGIYLAWYQQKPGKTFKLLIYSGSTLQSGTPSRFSGSGSGTDFTLTIRSLEPEDFGLYFCQQFYENPFTFGSGTKLEIRRA

SEQ ID NO: 31 - DNA, 327 bp, Rattus norvegicus
  source 1..327: mol_type = genomic DNA
gatgtccagatgacccagtctccgtcttctcttgctgcgtctcctggagaaagtgtttccatcagttgcagggcaactaagagcattggtatttatttagcctggtatcaacagaaacctgggaaaacatttaagcttcttatctactctgggtcaactttgcaatctggaactccatcaaggttcagtggcagtgggtctggtacagatttcactctcaccatcagaagcctggagcctgaagattttggactctatttctgtcaacagttttatgaaaacccattcacgttcggctcagggacgaagttggaaataagacgggct

SEQ ID NO: 32 - protein, 11 aa, Rattus norvegicus
RATKSIGIYLA

SEQ ID NO: 33 - protein, 7 aa, Rattus norvegicus
SGSTLQS

SEQ ID NO: 34 - protein, 9 aa, Rattus norvegicus
QQFYENPFT

SEQ ID NO: 35 - protein, 121 aa, Rattus norvegicus
EVQLQESGPGLVKPSQSLSLTCSVTDYSITTYFWGWIRKFPGNKMEWMGYMSYRGGTSYNPSLKSRISITRDTSKNQFFLQLNSVTTEDTATYYCARCPNYGGHSLVFDYWGQGVMVTVSS

SEQ ID NO: 36 - DNA, 363 bp, Rattus norvegicus
  source 1..363: mol_type = genomic DNA
gaggtgcagcttcaggagtcaggacctggccttgtgaaaccctcacagtcactctccctcacctgttctgtcactgattactccatcactacttatttctggggctggatccggaagttcccaggaaataaaatggagtggatgggatacatgagctaccgtggtggcacttcctacaacccatctctcaagagtcgaatctccattactagagacacatcgaagaatcagttcttcctgcagttgaactctgtaactactgaggacacagccacatattactgtgcaagatgccctaactacggagggcattcccttgtttttgattactggggccaaggagtcatggtcacagtgtcctca

SEQ ID NO: 37 - protein, 10 aa, Rattus norvegicus
DYSITTYFWG

SEQ ID NO: 38 - protein, 9 aa, Rattus norvegicus
YMSYRGGTS

SEQ ID NO: 39 - protein, 13 aa, Rattus norvegicus
CPNYGGHSLVFDY

SEQ ID NO: 40 - protein, 109 aa, Rattus norvegicus
DVQMTQSPSYLAASPGESVSISCKATKSISNYLAWYQQKPGEAYKVLIYSGSTLQSGTPSRFSGSGSGTDFTLTIRSLEPEDFGLYSCQQYYEKPLTFGSGTKLEIKRA

SEQ ID NO: 41 - DNA, 327 bp, Rattus norvegicus
  source 1..327: mol_type = genomic DNA
gatgtccagatgacccagtctccgtcttatcttgctgcgtctcctggagaaagtgtttccatcagttgcaaggcaactaagagcattagtaattatttagcctggtatcaacagaaacctggggaagcatataaggttcttatctattctgggtcaactttgcaatctggaactccatcaaggttcagtggcagtggatctggtacagatttcactctcaccatcagaagcctggagcctgaagattttggactctattcctgtcaacagtattatgaaaaaccgctcacgttcggttctgggaccaagctggagatcaaacgggct

SEQ ID NO: 42 - protein, 11 aa, Rattus norvegicus
KATKSISNYLA

SEQ ID NO: 43 - protein, 7 aa, Rattus norvegicus
SGSTLQS

SEQ ID NO: 44 - protein, 9 aa, Rattus norvegicus
QQYYEKPLT

SEQ ID NO: 45 - protein, 121 aa, Rattus norvegicus
EVQLQESGPGLVKPSQSLSLTCSVTGYSITTYYWGWIRKFPGNKMEWMGYISYSGRTSYNPSLKSRMSITRDASKNQFFLQLNSVTTDDTATYYCARSPINHGGYWYFDFWGPGTMVTVSS

SEQ ID NO: 46 - DNA, 363 bp, Rattus norvegicus
  source 1..363: mol_type = genomic DNA
gaggtgcagcttcaggagtcaggacctggccttgtgaaaccctcacagtcactctccctcacctgttctgtcactggttactccatcactacttattactggggctggatccggaagttcccaggaaataaaatggagtggatggggtacataagctacagtggtcgcactagttataacccatctctcaaaagtcgaatgtccattactagagacgcatcgaagaatcagttcttcctacagttgaactctgtaactactgacgacacagccacatattactgtgcaagatccccaattaaccacggagggtactggtactttgacttctggggcccaggaaccatggtcaccgtgtcctca

SEQ ID NO: 47 - protein, 10 aa, Rattus norvegicus
GYSITTYYWG

SEQ ID NO: 48 - protein, 9 aa, Rattus norvegicus
YISYSGRTS

SEQ ID NO: 49 - protein, 13 aa, Rattus norvegicus
SPINHGGYWYFDF

SEQ ID NO: 50 - DNA, 449 bp, synthetic construct
  misc_feature 1..449: note = DNA comprising DNA sequence coding for human light chain signal sequence and kappa chain constant region
  source 1..449: mol_type = other DNA
gcctccggactctagagccaccatggtgctgcagacccaggtgttcatctccctgctgctgtggatctccggcgcgtacggcgatatcgtgatgattaaacgtacggtggccgccccctccgtgttcatcttccccccctccgacgagcagctgaagtccggcaccgcctccgtggtgtgcctgctgaataacttctaccccagagaggccaaggtgcagtggaaggtggacaacgccctgcagtccgggaactcccaggagagcgtgaccgagcaggacagcaaggacagcacctacagcctgagcagcaccctgaccctgagcaaagccgactacgagaagcacaaggtgtacgcctgcgaggtgacccaccagggcctgagctcccccgtcaccaagagcttcaacaggggggagtgttaggggcccgtttaaacgggggaggcta

SEQ ID NO: 51 - DNA, 1132 bp, synthetic construct
  misc_feature 1..1132: note = DNA comprising DNA sequence coding for human heavy chain signal sequence and IgG1 constant region
  source 1..1132: mol_type = other DNA
gcctccggactctagagccaccatgaaacacctgtggttcttcctcctgctggtggcagctcccagatgggtgctgagccaggtgcaattgtgcaggcggttagctcagcctccaccaagggcccaagcgtcttccccctggcaccctcctccaagagcacctctggcggcacagccgccctgggctgcctggtcaaggactacttccccgaacccgtgaccgtgagctggaactcaggcgccctgaccagcggcgtgcacaccttccccgctgtcctgcagtcctcaggactctactccctcagcagcgtggtgaccgtgccctccagcagcttgggcacccagacctacatctgcaacgtgaatcacaagcccagcaacaccaaggtggacaagagagttgagcccaaatcttgtgacaaaactcacacatgcccaccctgcccagcacctgaactcctggggggaccctcagtcttcctcttccccccaaaacccaaggacaccctcatgatctcccggacccctgaggtcacatgcgtggtggtggacgtgagccacgaagaccctgaggtcaagttcaactggtacgtggacggcgtggaggtgcataatgccaagacaaagccccgggaggagcagtacaacagcacgtaccgggtggtcagcgtcctcaccgtcctgcaccaggactggctgaatggcaaggagtacaagtgcaaggtctccaacaaagccctcccagcccccatcgagaaaaccatctccaaagccaaaggccagccccgggaaccacaggtgtacaccctgcccccatcccgggaggagatgaccaagaaccaggtcagcctgacctgcctggtcaaaggcttctatcccagcgacatcgccgtggagtgggagagcaatggccagcccgagaacaactacaagaccacccctcccgtgctggactccgacggctccttcttcctctacagcaagctcaccgtggacaagagcaggtggcagcagggcaacgtcttctcatgctccgtgatgcatgaggctctgcacaaccactacacccagaagagcctctccctgtctcccggcaaatgagatatcgggcccgtttaaacgggggaggcta

SEQ ID NO: 52 - DNA, 749 bp, synthetic construct
  misc_feature 1..749: note = DNA comprising DNA sequence coding for chG019 light chain
  source 1..749: mol_type = other DNA
ccagcctccggactctagagccaccatggtgctgcagacccaggtgttcatcagcctgctgctgtggatcagcggcgcctacggcgacatccagatgacccagagccctagcctgctgagcgccagcgtgggcgatagagtgaccctgaactgcaaggccagccagaacatctacaagaacctggcctggtatcagcagaagctgggcgagggccccaagctgctgatctacgacgccaacaccctgcagaccggcatccccagcagattttctggcagcggcagcggctccgacttcaccctgacaatcagcagcctgcagcccgaggacgtggccacctacttttgccagcagtactacagcggctgggccttcggcggcgtgaccaacctggaactgaagagagccgtggccgctccctccgtgttcatcttcccacctagcgacgagcagctgaagtccggcacagcctctgtcgtgtgcctgctgaacaacttctacccccgcgaggccaaggtgcagtggaaggtggacaatgccctgcagtctggcaacagccaggaaagcgtgaccgagcaggacagcaaggactccacctacagcctgagcagcaccctgaccctgagcaaggccgactacgagaagcacaaggtgtacgcctgcgaagtgacccaccagggcctgtctagccccgtgaccaagagcttcaaccggggcgagtgttgagtttaaacgggggaggctaact

SEQ ID NO: 53 - protein, 233 aa, synthetic construct
  REGION 1..233: note = amino acid sequesnce of chG019 light chain full-length
MVLQTQVFISLLLWISGAYGDIQMTQSPSLLSASVGDRVTLNCKASQNIYKNLAWYQQKLGEGPKLLIYDANTLQTGIPSRFSGSGSGSDFTLTISSLQPEDVATYFCQQYYSGWAFGGVTNLELKRAVAAPSVFIFPPSDEQLKSGTASVVCLLNNFYPREAKVQWKVDNALQSGNSQESVTEQDSKDSTYSLSSTLTLSKADYEKHKVYACEVTHQGLSSPVTKSFNRGEC

SEQ ID NO: 54 - DNA, 699 bp, synthetic construct
  misc_feature 1..699: note = nucleotide sequesnce of chG019 light chain full-length
  source 1..699: mol_type = other DNA
atggtgctgcagacccaggtgttcatcagcctgctgctgtggatcagcggcgcctacggcgacatccagatgacccagagccctagcctgctgagcgccagcgtgggcgatagagtgaccctgaactgcaaggccagccagaacatctacaagaacctggcctggtatcagcagaagctgggcgagggccccaagctgctgatctacgacgccaacaccctgcagaccggcatccccagcagattttctggcagcggcagcggctccgacttcaccctgacaatcagcagcctgcagcccgaggacgtggccacctacttttgccagcagtactacagcggctgggccttcggcggcgtgaccaacctggaactgaagagagccgtggccgctccctccgtgttcatcttcccacctagcgacgagcagctgaagtccggcacagcctctgtcgtgtgcctgctgaacaacttctacccccgcgaggccaaggtgcagtggaaggtggacaatgccctgcagtctggcaacagccaggaaagcgtgaccgagcaggacagcaaggactccacctacagcctgagcagcaccctgaccctgagcaaggccgactacgagaagcacaaggtgtacgcctgcgaagtgacccaccagggcctgtctagccccgtgaccaagagcttcaaccggggcgagtgt

SEQ ID NO: 55 - DNA, 324 bp, synthetic construct
  misc_feature 1..324: note = nucleotide sequesnce of chG019 light chain variable region
  source 1..324: mol_type = other DNA
gacatccagatgacccagagccctagcctgctgagcgccagcgtgggcgatagagtgaccctgaactgcaaggccagccagaacatctacaagaacctggcctggtatcagcagaagctgggcgagggccccaagctgctgatctacgacgccaacaccctgcagaccggcatccccagcagattttctggcagcggcagcggctccgacttcaccctgacaatcagcagcctgcagcccgaggacgtggccacctacttttgccagcagtactacagcggctgggccttcggcggcgtgaccaacctggaactgaagagagcc

SEQ ID NO: 56 - protein, 471 aa, synthetic construct
  REGION 1..471: note = amino acid sequesnce of chG019 heavy chain full-length
MKHLWFFLLLVAAPRWVLSQVQLQQSGAELVKPGSSVKISCKASGYTFTRNFMHWIKQQPGNGLEWIGWIYPGDGETEYNQKFNGKATLTADRSSSTAYMELSRLTSEDSAVYFCARGVYGGFAGGYFDFWGQGVMVTVSSASTKGPSVFPLAPSSKSTSGGTAALGCLVKDYFPEPVTVSWNSGALTSGVHTFPAVLQSSGLYSLSSVVTVPSSSLGTQTYICNVNHKPSNTKVDKRVEPKSCDKTHTCPPCPAPELLGGPSVFLFPPKPKDTLMISRTPEVTCVVVDVSHEDPEVKFNWYVDGVEVHNAKTKPREEQYNSTYRVVSVLTVLHQDWLNGKEYKCKVSNKALPAPIEKTISKAKGQPREPQVYTLPPSREEMTKNQVSLTCLVKGFYPSDIAVEWESNGQPENNYKTTPPVLDSDGSFFLYSKLTVDKSRWQQGNVFSCSVMHEALHNHYTQKSLSLSPGK

SEQ ID NO: 57 - DNA, 1413 bp, synthetic construct
  misc_feature 1..1413: note = nucleotide sequesnce of chG019 heavy chain full-length
  source 1..1413: mol_type = other DNA
atgaaacacctgtggttcttcctcctgctggtggcagctcccagatgggtgctgagccaggtgcagctgcagcagtctggcgccgagctcgtgaagcctggcagcagcgtgaagatcagctgcaaggccagcggctacaccttcacccggaacttcatgcactggatcaagcagcagcccggcaacggcctggaatggatcggctggatctatcccggcgacggcgagacagagtacaaccagaagttcaacggcaaggccaccctgaccgccgacagaagcagctccaccgcctacatggaactgagccggctgaccagcgaggacagcgccgtgtacttttgcgccagaggcgtgtacggcggcttcgctggcggctacttcgatttttggggccagggcgtgatggtcaccgtcagctcagcctccaccaagggcccaagcgtcttccccctggcaccctcctccaagagcacctctggcggcacagccgccctgggctgcctggtcaaggactacttccccgaacccgtgaccgtgagctggaactcaggcgccctgaccagcggcgtgcacaccttccccgctgtcctgcagtcctcaggactctactccctcagcagcgtggtgaccgtgccctccagcagcttgggcacccagacctacatctgcaacgtgaatcacaagcccagcaacaccaaggtggacaagagagttgagcccaaatcttgtgacaaaactcacacatgcccaccctgcccagcacctgaactcctggggggaccctcagtcttcctcttccccccaaaacccaaggacaccctcatgatctcccggacccctgaggtcacatgcgtggtggtggacgtgagccacgaagaccctgaggtcaagttcaactggtacgtggacggcgtggaggtgcataatgccaagacaaagccccgggaggagcagtacaacagcacgtaccgggtggtcagcgtcctcaccgtcctgcaccaggactggctgaatggcaaggagtacaagtgcaaggtctccaacaaagccctcccagcccccatcgagaaaaccatctccaaagccaaaggccagccccgggaaccacaggtgtacaccctgcccccatcccgggaggagatgaccaagaaccaggtcagcctgacctgcctggtcaaaggcttctatcccagcgacatcgccgtggagtgggagagcaatggccagcccgagaacaactacaagaccacccctcccgtgctggactccgacggctccttcttcctctacagcaagctcaccgtggacaagagcaggtggcagcagggcaacgtcttctcatgctccgtgatgcatgaggctctgcacaaccactacacccagaagagcctctccctgtctcccggcaaa

SEQ ID NO: 58 - protein, 122 aa, synthetic construct
  REGION 1..122: note = amino acid sequesnce of chG019 heavy chain variable region
QVQLQQSGAELVKPGSSVKISCKASGYTFTRNFMHWIKQQPGNGLEWIGWIYPGDGETEYNQKFNGKATLTADRSSSTAYMELSRLTSEDSAVYFCARGVYGGFAGGYFDFWGQGVMVTVSS

SEQ ID NO: 59 - DNA, 366 bp, synthetic construct
  misc_feature 1..366: note = nucleotide sequesnce of chG019 heavy chain variable region
  source 1..366: mol_type = other DNA
caggtgcagctgcagcagtctggcgccgagctcgtgaagcctggcagcagcgtgaagatcagctgcaaggccagcggctacaccttcacccggaacttcatgcactggatcaagcagcagcccggcaacggcctggaatggatcggctggatctatcccggcgacggcgagacagagtacaaccagaagttcaacggcaaggccaccctgaccgccgacagaagcagctccaccgcctacatggaactgagccggctgaccagcgaggacagcgccgtgtacttttgcgccagaggcgtgtacggcggcttcgctggcggctacttcgatttttggggccagggcgtgatggtcaccgtcagctca

SEQ ID NO: 60 - protein, 10 aa, synthetic construct
  REGION 1..10: note = amino acid sequesnce of chG019 CDRH2
WIYPGDGETE

SEQ ID NO: 61 - protein, 233 aa, synthetic construct
  REGION 1..233: note = amino acid sequesnce of hL02 light chain full-length
MVLQTQVFISLLLWISGAYGDIQMTQSPSSLSASVGDRVTITCKASQNIYKNLAWYQQKPGKAPKLLIYDANTLQTGVPSRFSGSGSGSDFTLTISSLQPEDFATYFCQQYYSGWAFGQGTKVEIKRTVAAPSVFIFPPSDEQLKSGTASVVCLLNNFYPREAKVQWKVDNALQSGNSQESVTEQDSKDSTYSLSSTLTLSKADYEKHKVYACEVTHQGLSSPVTKSFNRGEC

SEQ ID NO: 62 - DNA, 699 bp, synthetic construct
  misc_feature 1..699: note = nucleotide sequesnce of hL02 light chain full-length
  source 1..699: mol_type = other DNA
atggtgctgcagacccaggtgttcatctccctgctgctgtggatctccggcgcgtacggcgacatccagatgacccagagccctagcagcctgagcgccagcgtgggcgacagagtgaccatcacatgcaaggccagccagaacatctacaagaacctggcctggtatcagcagaagcccggcaaggcccccaagctgctgatctacgacgccaacaccctgcagaccggcgtgcccagcagattttctggcagcggcagcggctccgacttcaccctgacaatcagcagcctgcagcccgaggacttcgccacctacttttgccagcagtactacagcggctgggccttcggccagggcaccaaggtggaaatcaagcgtacggtggccgccccctccgtgttcatcttccccccctccgacgagcagctgaagtccggcaccgcctccgtggtgtgcctgctgaataacttctaccccagagaggccaaggtgcagtggaaggtggacaacgccctgcagtccgggaactcccaggagagcgtgaccgagcaggacagcaaggacagcacctacagcctgagcagcaccctgaccctgagcaaagccgactacgagaagcacaaggtgtacgcctgcgaggtgacccaccagggcctgagctcccccgtcaccaagagcttcaacaggggggagtgt

SEQ ID NO: 63 - protein, 108 aa, synthetic construct
  REGION 1..108: note = amino acid sequesnce of hL02 light chain variable region
DIQMTQSPSSLSASVGDRVTITCKASQNIYKNLAWYQQKPGKAPKLLIYDANTLQTGVPSRFSGSGSGSDFTLTISSLQPEDFATYFCQQYYSGWAFGQGTKVEIKRT

SEQ ID NO: 64 - DNA, 324 bp, synthetic construct
  misc_feature 1..324: note = nucleotide sequesnce of hL02 light chain variable region
  source 1..324: mol_type = other DNA
gacatccagatgacccagagccctagcagcctgagcgccagcgtgggcgacagagtgaccatcacatgcaaggccagccagaacatctacaagaacctggcctggtatcagcagaagcccggcaaggcccccaagctgctgatctacgacgccaacaccctgcagaccggcgtgcccagcagattttctggcagcggcagcggctccgacttcaccctgacaatcagcagcctgcagcccgaggacttcgccacctacttttgccagcagtactacagcggctgggccttcggccagggcaccaaggtggaaatcaagcgtacg

SEQ ID NO: 65 - protein, 233 aa, synthetic construct
  REGION 1..233: note = amino acid sequesnce of hL03 light chain full-length
MVLQTQVFISLLLWISGAYGDIQMTQSPSSLSASVGDRVTITCKASQNIYKNLAWYQQKLGEGPKLLIYDANTLQTGVPSRFSGSGSGTDFTLTISSLQPEDFATYYCQQYYSGWAFGQGTKVEIKRTVAAPSVFIFPPSDEQLKSGTASVVCLLNNFYPREAKVQWKVDNALQSGNSQESVTEQDSKDSTYSLSSTLTLSKADYEKHKVYACEVTHQGLSSPVTKSFNRGEC

SEQ ID NO: 66 - DNA, 699 bp, synthetic construct
  misc_feature 1..699: note = nucleotide sequesnce of hL03 light chain full-length
  source 1..699: mol_type = other DNA
atggtgctgcagacccaggtgttcatctccctgctgctgtggatctccggcgcgtacggcgacatccagatgacccagagccctagcagcctgagcgccagcgtgggcgacagagtgaccatcacatgcaaggccagccagaacatctacaagaacctggcctggtatcagcagaagctgggcgagggccccaagctgctgatctacgacgccaacaccctgcagaccggcgtgcccagcagattttctggcagcggctccggcaccgacttcaccctgacaatcagcagcctgcagcccgaggacttcgccacctactactgccagcagtactacagcggctgggcctttggccagggcaccaaggtggaaatcaagcgtacggtggccgccccctccgtgttcatcttccccccctccgacgagcagctgaagtccggcaccgcctccgtggtgtgcctgctgaataacttctaccccagagaggccaaggtgcagtggaaggtggacaacgccctgcagtccgggaactcccaggagagcgtgaccgagcaggacagcaaggacagcacctacagcctgagcagcaccctgaccctgagcaaagccgactacgagaagcacaaggtgtacgcctgcgaggtgacccaccagggcctgagctcccccgtcaccaagagcttcaacaggggggagtgt

SEQ ID NO: 67 - protein, 108 aa, synthetic construct
  REGION 1..108: note = amino acid sequesnce of hL03 light chain variable region
DIQMTQSPSSLSASVGDRVTITCKASQNIYKNLAWYQQKLGEGPKLLIYDANTLQTGVPSRFSGSGSGTDFTLTISSLQPEDFATYYCQQYYSGWAFGQGTKVEIKRT

SEQ ID NO: 68 - DNA, 324 bp, synthetic construct
  misc_feature 1..324: note = nucleotide sequesnce of hL03 light chain variable region
  source 1..324: mol_type = other DNA
gacatccagatgacccagagccctagcagcctgagcgccagcgtgggcgacagagtgaccatcacatgcaaggccagccagaacatctacaagaacctggcctggtatcagcagaagctgggcgagggccccaagctgctgatctacgacgccaacaccctgcagaccggcgtgcccagcagattttctggcagcggctccggcaccgacttcaccctgacaatcagcagcctgcagcccgaggacttcgccacctactactgccagcagtactacagcggctgggcctttggccagggcaccaaggtggaaatcaagcgtacg

SEQ ID NO: 69 - protein, 471 aa, synthetic construct
  REGION 1..471: note = amino acid sequesnce of hH01 heavy chain full-length
MKHLWFFLLLVAAPRWVLSEVQLVQSGAEVKKPGASVKVSCKASGYTFTRNFMHWVRQAPGQGLEWMGWIYPGDGETEYAQKFQGRVTITADTSTSTAYMELSSLRSEDTAVYYCARGVYGGFAGGYFDFWGQGTLVTVSSASTKGPSVFPLAPSSKSTSGGTAALGCLVKDYFPEPVTVSWNSGALTSGVHTFPAVLQSSGLYSLSSVVTVPSSSLGTQTYICNVNHKPSNTKVDKRVEPKSCDKTHTCPPCPAPELLGGPSVFLFPPKPKDTLMISRTPEVTCVVVDVSHEDPEVKFNWYVDGVEVHNAKTKPREEQYNSTYRVVSVLTVLHQDWLNGKEYKCKVSNKALPAPIEKTISKAKGQPREPQVYTLPPSREEMTKNQVSLTCLVKGFYPSDIAVEWESNGQPENNYKTTPPVLDSDGSFFLYSKLTVDKSRWQQGNVFSCSVMHEALHNHYTQKSLSLSPGK

SEQ ID NO: 70 - DNA, 1413 bp, synthetic construct
  misc_feature 1..1413: note = nucleotide sequesnce of hH01 heavy chain full-length
  source 1..1413: mol_type = other DNA
atgaaacacctgtggttcttcctcctgctggtggcagctcccagatgggtgctgagcgaagtgcagctggtgcagtctggcgccgaagtgaagaaaccaggcgccagcgtgaaggtgtcctgcaaggccagcggctacacctttacccggaacttcatgcactgggtgcgccaggctccaggccagggactggaatggatgggctggatctatcccggcgacggcgagacagagtacgcccagaaattccagggcagagtgaccatcaccgccgacaccagcacctccaccgcctacatggaactgagcagcctgcggagcgaggacaccgccgtgtactattgtgccagaggcgtgtacggcggcttcgctggcggctacttcgatttttggggccagggcaccctcgtgaccgtcagctcagcctccaccaagggcccaagcgtcttccccctggcaccctcctccaagagcacctctggcggcacagccgccctgggctgcctggtcaaggactacttccccgaacccgtgaccgtgagctggaactcaggcgccctgaccagcggcgtgcacaccttccccgctgtcctgcagtcctcaggactctactccctcagcagcgtggtgaccgtgccctccagcagcttgggcacccagacctacatctgcaacgtgaatcacaagcccagcaacaccaaggtggacaagagagttgagcccaaatcttgtgacaaaactcacacatgcccaccctgcccagcacctgaactcctggggggaccctcagtcttcctcttccccccaaaacccaaggacaccctcatgatctcccggacccctgaggtcacatgcgtggtggtggacgtgagccacgaagaccctgaggtcaagttcaactggtacgtggacggcgtggaggtgcataatgccaagacaaagccccgggaggagcagtacaacagcacgtaccgggtggtcagcgtcctcaccgtcctgcaccaggactggctgaatggcaaggagtacaagtgcaaggtctccaacaaagccctcccagcccccatcgagaaaaccatctccaaagccaaaggccagccccgggaaccacaggtgtacaccctgcccccatcccgggaggagatgaccaagaaccaggtcagcctgacctgcctggtcaaaggcttctatcccagcgacatcgccgtggagtgggagagcaatggccagcccgagaacaactacaagaccacccctcccgtgctggactccgacggctccttcttcctctacagcaagctcaccgtggacaagagcaggtggcagcagggcaacgtcttctcatgctccgtgatgcatgaggctctgcacaaccactacacccagaagagcctctccctgtctcccggcaaa

SEQ ID NO: 71 - protein, 122 aa, synthetic construct
  REGION 1..122: note = amino acid sequesnce of hH01 heavy chain variable region
EVQLVQSGAEVKKPGASVKVSCKASGYTFTRNFMHWVRQAPGQGLEWMGWIYPGDGETEYAQKFQGRVTITADTSTSTAYMELSSLRSEDTAVYYCARGVYGGFAGGYFDFWGQGTLVTVSS

SEQ ID NO: 72 - DNA, 366 bp, synthetic construct
  misc_feature 1..366: note = nucleotide sequesnce of hH01 heavy chain variable region
  source 1..366: mol_type = other DNA
gaagtgcagctggtgcagtctggcgccgaagtgaagaaaccaggcgccagcgtgaaggtgtcctgcaaggccagcggctacacctttacccggaacttcatgcactgggtgcgccaggctccaggccagggactggaatggatgggctggatctatcccggcgacggcgagacagagtacgcccagaaattccagggcagagtgaccatcaccgccgacaccagcacctccaccgcctacatggaactgagcagcctgcggagcgaggacaccgccgtgtactattgtgccagaggcgtgtacggcggcttcgctggcggctacttcgatttttggggccagggcaccctcgtgaccgtcagctca

SEQ ID NO: 73 - protein, 471 aa, synthetic construct
  REGION 1..471: note = amino acid sequesnce of hH02 heavy chain full-length
MKHLWFFLLLVAAPRWVLSEVQLVQSGAEVKKPGASVKVSCKASGYTFTRNFMHWVRQAPGQGLEWMGWIYPGDGETEYNQKFQGRVTITADRSTSTAYMELSSLRSEDTAVYFCARGVYGGFAGGYFDFWGQGTLVTVSSASTKGPSVFPLAPSSKSTSGGTAALGCLVKDYFPEPVTVSWNSGALTSGVHTFPAVLQSSGLYSLSSVVTVPSSSLGTQTYICNVNHKPSNTKVDKRVEPKSCDKTHTCPPCPAPELLGGPSVFLFPPKPKDTLMISRTPEVTCVVVDVSHEDPEVKFNWYVDGVEVHNAKTKPREEQYNSTYRVVSVLTVLHQDWLNGKEYKCKVSNKALPAPIEKTISKAKGQPREPQVYTLPPSREEMTKNQVSLTCLVKGFYPSDIAVEWESNGQPENNYKTTPPVLDSDGSFFLYSKLTVDKSRWQQGNVFSCSVMHEALHNHYTQKSLSLSPGK

SEQ ID NO: 74 - DNA, 1413 bp, synthetic construct
  misc_feature 1..1413: note = nucleotide sequesnce of hH02 heavy chain full-length
  source 1..1413: mol_type = other DNA
atgaaacacctgtggttcttcctcctgctggtggcagctcccagatgggtgctgagcgaagtgcagctggtgcagtctggcgccgaagtgaagaaaccaggcgccagcgtgaaggtgtcctgcaaggccagcggctacacctttacccggaacttcatgcactgggtgcgccaggctccaggccagggactggaatggatgggctggatctatcccggcgacggcgagacagagtacaaccagaaattccagggcagagtgaccatcaccgccgacagaagcaccagcaccgcctacatggaactgagcagcctgcggagcgaggataccgccgtgtacttctgtgccagaggcgtgtacggcggcttcgctggcggctacttcgatttttggggccagggcaccctcgtgaccgtcagctcagcctccaccaagggcccaagcgtcttccccctggcaccctcctccaagagcacctctggcggcacagccgccctgggctgcctggtcaaggactacttccccgaacccgtgaccgtgagctggaactcaggcgccctgaccagcggcgtgcacaccttccccgctgtcctgcagtcctcaggactctactccctcagcagcgtggtgaccgtgccctccagcagcttgggcacccagacctacatctgcaacgtgaatcacaagcccagcaacaccaaggtggacaagagagttgagcccaaatcttgtgacaaaactcacacatgcccaccctgcccagcacctgaactcctggggggaccctcagtcttcctcttccccccaaaacccaaggacaccctcatgatctcccggacccctgaggtcacatgcgtggtggtggacgtgagccacgaagaccctgaggtcaagttcaactggtacgtggacggcgtggaggtgcataatgccaagacaaagccccgggaggagcagtacaacagcacgtaccgggtggtcagcgtcctcaccgtcctgcaccaggactggctgaatggcaaggagtacaagtgcaaggtctccaacaaagccctcccagcccccatcgagaaaaccatctccaaagccaaaggccagccccgggaaccacaggtgtacaccctgcccccatcccgggaggagatgaccaagaaccaggtcagcctgacctgcctggtcaaaggcttctatcccagcgacatcgccgtggagtgggagagcaatggccagcccgagaacaactacaagaccacccctcccgtgctggactccgacggctccttcttcctctacagcaagctcaccgtggacaagagcaggtggcagcagggcaacgtcttctcatgctccgtgatgcatgaggctctgcacaaccactacacccagaagagcctctccctgtctcccggcaaa

SEQ ID NO: 75 - protein, 122 aa, synthetic construct
  REGION 1..122: note = amino acid sequesnce of hH02 heavy chain variable region
EVQLVQSGAEVKKPGASVKVSCKASGYTFTRNFMHWVRQAPGQGLEWMGWIYPGDGETEYNQKFQGRVTITADRSTSTAYMELSSLRSEDTAVYFCARGVYGGFAGGYFDFWGQGTLVTVSS

SEQ ID NO: 76 - DNA, 366 bp, synthetic construct
  misc_feature 1..366: note = nucleotide sequesnce of hH02 heavy chain variable region
  source 1..366: mol_type = other DNA
gaagtgcagctggtgcagtctggcgccgaagtgaagaaaccaggcgccagcgtgaaggtgtcctgcaaggccagcggctacacctttacccggaacttcatgcactgggtgcgccaggctccaggccagggactggaatggatgggctggatctatcccggcgacggcgagacagagtacaaccagaaattccagggcagagtgaccatcaccgccgacagaagcaccagcaccgcctacatggaactgagcagcctgcggagcgaggataccgccgtgtacttctgtgccagaggcgtgtacggcggcttcgctggcggctacttcgatttttggggccagggcaccctcgtgaccgtcagctca

SEQ ID NO: 77 - protein, 471 aa, synthetic construct
  REGION 1..471: note = amino acid sequesnce of hH04 heavy chain full-length
MKHLWFFLLLVAAPRWVLSQVQLVQSGAEVKKPGASVKVSCKASGYTFTRNFMHWIRQAPGQGLEWMGWIYPGDGETEYAQKFQGRVTLTADRSTSTAYMELSSLRSEDTAVYYCARGVYGGFAGGYFDFWGQGTLVTVSSASTKGPSVFPLAPSSKSTSGGTAALGCLVKDYFPEPVTVSWNSGALTSGVHTFPAVLQSSGLYSLSSVVTVPSSSLGTQTYICNVNHKPSNTKVDKRVEPKSCDKTHTCPPCPAPELLGGPSVFLFPPKPKDTLMISRTPEVTCVVVDVSHEDPEVKFNWYVDGVEVHNAKTKPREEQYNSTYRVVSVLTVLHQDWLNGKEYKCKVSNKALPAPIEKTISKAKGQPREPQVYTLPPSREEMTKNQVSLTCLVKGFYPSDIAVEWESNGQPENNYKTTPPVLDSDGSFFLYSKLTVDKSRWQQGNVFSCSVMHEALHNHYTQKSLSLSPGK

SEQ ID NO: 78 - DNA, 1413 bp, synthetic construct
  misc_feature 1..1413: note = nucleotide sequesnce of hH04 heavy chain full-length
  source 1..1413: mol_type = other DNA
atgaaacacctgtggttcttcctcctgctggtggcagctcccagatgggtgctgagccaggtgcagctggtgcagtctggcgccgaagtgaagaaaccaggcgccagcgtgaaggtgtcctgcaaggccagcggctacacctttacccggaacttcatgcactggatccggcaggcccctggacagggcctggaatggatgggctggatctatcccggcgacggcgagacagagtacgcccagaaattccagggcagagtgaccctgaccgccgacagaagcaccagcaccgcctacatggaactgagcagcctgcggagcgaggacaccgccgtgtactattgtgccagaggcgtgtacggcggcttcgctggcggctacttcgatttttggggccagggcaccctcgtgaccgtcagctcagcctccaccaagggcccaagcgtcttccccctggcaccctcctccaagagcacctctggcggcacagccgccctgggctgcctggtcaaggactacttccccgaacccgtgaccgtgagctggaactcaggcgccctgaccagcggcgtgcacaccttccccgctgtcctgcagtcctcaggactctactccctcagcagcgtggtgaccgtgccctccagcagcttgggcacccagacctacatctgcaacgtgaatcacaagcccagcaacaccaaggtggacaagagagttgagcccaaatcttgtgacaaaactcacacatgcccaccctgcccagcacctgaactcctggggggaccctcagtcttcctcttccccccaaaacccaaggacaccctcatgatctcccggacccctgaggtcacatgcgtggtggtggacgtgagccacgaagaccctgaggtcaagttcaactggtacgtggacggcgtggaggtgcataatgccaagacaaagccccgggaggagcagtacaacagcacgtaccgggtggtcagcgtcctcaccgtcctgcaccaggactggctgaatggcaaggagtacaagtgcaaggtctccaacaaagccctcccagcccccatcgagaaaaccatctccaaagccaaaggccagccccgggaaccacaggtgtacaccctgcccccatcccgggaggagatgaccaagaaccaggtcagcctgacctgcctggtcaaaggcttctatcccagcgacatcgccgtggagtgggagagcaatggccagcccgagaacaactacaagaccacccctcccgtgctggactccgacggctccttcttcctctacagcaagctcaccgtggacaagagcaggtggcagcagggcaacgtcttctcatgctccgtgatgcatgaggctctgcacaaccactacacccagaagagcctctccctgtctcccggcaaa

SEQ ID NO: 79 - protein, 122 aa, synthetic construct
  REGION 1..122: note = amino acid sequesnce of hH04 heavy chain variable region
QVQLVQSGAEVKKPGASVKVSCKASGYTFTRNFMHWIRQAPGQGLEWMGWIYPGDGETEYAQKFQGRVTLTADRSTSTAYMELSSLRSEDTAVYYCARGVYGGFAGGYFDFWGQGTLVTVSS

SEQ ID NO: 80 - DNA, 366 bp, synthetic construct
  misc_feature 1..366: note = nucleotide sequesnce of hH04 heavy chain variable region
  source 1..366: mol_type = other DNA
caggtgcagctggtgcagtctggcgccgaagtgaagaaaccaggcgccagcgtgaaggtgtcctgcaaggccagcggctacacctttacccggaacttcatgcactggatccggcaggcccctggacagggcctggaatggatgggctggatctatcccggcgacggcgagacagagtacgcccagaaattccagggcagagtgaccctgaccgccgacagaagcaccagcaccgcctacatggaactgagcagcctgcggagcgaggacaccgccgtgtactattgtgccagaggcgtgtacggcggcttcgctggcggctacttcgatttttggggccagggcaccctcgtgaccgtcagctca

SEQ ID NO: 81 - protein, 235 aa, synthetic construct
  REGION 1..235: note = amino acid sequesnce of NOV0712 light chain full-length
MVLQTQVFISLLLWISGAYGDIQMTQSPSSLSASVGDRVTITCRASQSISSYLNWYQQKPGKAPKLLIYAVSTLQSGVPSRFSGSGSGTDFTLTISSLQPEDFATYYCQQSGTFPPTTFGQGTKVEIKRTVAAPSVFIFPPSDEQLKSGTASVVCLLNNFYPREAKVQWKVDNALQSGNSQESVTEQDSKDSTYSLSSTLTLSKADYEKHKVYACEVTHQGLSSPVTKSFNRGEC

SEQ ID NO: 82 - DNA, 705 bp, synthetic construct
  misc_feature 1..705: note = nucleotide sequesnce coding for amino acid sequence of sequence number 81
  source 1..705: mol_type = other DNA
atggtgctgcagacccaggtgttcatctccctgctgctgtggatctccggcgcgtacggcgacatccagatgacccagagccctagcagcctgagcgccagcgtgggcgacagagtgaccatcacctgtagagccagccagagcatcagcagctacctgaactggtatcagcagaagcccggcaaggcccccaaactgctgatctacgccgtgtccacactgcagagcggcgtgcccagcagattttctggcagcggctccggcaccgacttcaccctgacaatcagcagcctgcagcccgaggacttcgccacctactactgtcagcagtccggcaccttcccccccaccacatttggccagggcaccaaggtggaaatcaagcgtacggtggccgccccctccgtgttcatcttccccccctccgacgagcagctgaagtccggcaccgcctccgtggtgtgcctgctgaataacttctaccccagagaggccaaggtgcagtggaaggtggacaacgccctgcagtccgggaactcccaggagagcgtgaccgagcaggacagcaaggacagcacctacagcctgagcagcaccctgaccctgagcaaagccgactacgagaagcacaaggtgtacgcctgcgaggtgacccaccagggcctgagctcccccgtcaccaagagcttcaacaggggggagtgt

SEQ ID NO: 83 - protein, 467 aa, synthetic construct
  REGION 1..467: note = amino acid sequesnce of NOV0712 heavy chain full-length
MKHLWFFLLLVAAPRWVLSQVQLLESGGGLVQPGGSLRLSCAASGFTFSSHGMHWVRQAPGKGLEWVSVISGSGSNTGYADSVKGRFTISRDNSKNTLYLQMNSLRAEDTAVYYCARQWGSYAFDSWGQGTLVTVSSASTKGPSVFPLAPSSKSTSGGTAALGCLVKDYFPEPVTVSWNSGALTSGVHTFPAVLQSSGLYSLSSVVTVPSSSLGTQTYICNVNHKPSNTKVDKRVEPKSCDKTHTCPPCPAPELLGGPSVFLFPPKPKDTLMISRTPEVTCVVVDVSHEDPEVKFNWYVDGVEVHNAKTKPREEQYNSTYRVVSVLTVLHQDWLNGKEYKCKVSNKALPAPIEKTISKAKGQPREPQVYTLPPSREEMTKNQVSLTCLVKGFYPSDIAVEWESNGQPENNYKTTPPVLDSDGSFFLYSKLTVDKSRWQQGNVFSCSVMHEALHNHYTQKSLSLSPGK

SEQ ID NO: 84 - DNA, 1401 bp, synthetic construct
  misc_feature 1..1401: note = nucleotide sequesnce coding for amino acid sequence of sequence number 83
  source 1..1401: mol_type = other DNA
atgaaacacctgtggttcttcctcctgctggtggcagctcccagatgggtgctgagccaggtgcagctgctggaatctggcggaggactggtgcagcctggcggctctctgagactgtcttgtgccgccagcggcttcaccttcagcagccacggaatgcactgggtgcgccaggcccctggaaagggactggaatgggtgtccgtgatcagcggcagcggctccaataccggctacgccgatagcgtgaagggccggttcaccatcagccgggacaacagcaagaacaccctgtacctgcagatgaacagcctgcgggccgaggacaccgccgtgtactattgtgccagacagtggggcagctacgccttcgattcttggggccagggcaccctcgtgaccgtcagctcagcctccaccaagggcccaagcgtcttccccctggcaccctcctccaagagcacctctggcggcacagccgccctgggctgcctggtcaaggactacttccccgaacccgtgaccgtgagctggaactcaggcgccctgaccagcggcgtgcacaccttccccgctgtcctgcagtcctcaggactctactccctcagcagcgtggtgaccgtgccctccagcagcttgggcacccagacctacatctgcaacgtgaatcacaagcccagcaacaccaaggtggacaagagagttgagcccaaatcttgtgacaaaactcacacatgcccaccctgcccagcacctgaactcctggggggaccctcagtcttcctcttccccccaaaacccaaggacaccctcatgatctcccggacccctgaggtcacatgcgtggtggtggacgtgagccacgaagaccctgaggtcaagttcaactggtacgtggacggcgtggaggtgcataatgccaagacaaagccccgggaggagcagtacaacagcacgtaccgggtggtcagcgtcctcaccgtcctgcaccaggactggctgaatggcaaggagtacaagtgcaaggtctccaacaaagccctcccagcccccatcgagaaaaccatctccaaagccaaaggccagccccgggaaccacaggtgtacaccctgcccccatcccgggaggagatgaccaagaaccaggtcagcctgacctgcctggtcaaaggcttctatcccagcgacatcgccgtggagtgggagagcaatggccagcccgagaacaactacaagaccacccctcccgtgctggactccgacggctccttcttcctctacagcaagctcaccgtggacaagagcaggtggcagcagggcaacgtcttctcatgctccgtgatgcatgaggctctgcacaaccactacacccagaagagcctctccctgtctcccggcaaa

SEQ ID NO: 85 - DNA, 34 bp, synthetic construct
  misc_feature 1..34: note = primer
  source 1..34: mol_type = other DNA
caccatgagaacttaccgctacttcttgctgctc

SEQ ID NO: 86 - DNA, 30 bp, synthetic construct
  misc_feature 1..30: note = primer
  source 1..30: mol_type = other DNA
ttaggagtctttgtcactgtccactcctcc